European Patent Application EP 4 755 391 A1, published June 10, 2026. Title: Therapy of Parkinson's Disease and Multiple System Atrophy. Applicant: HUN-REN Természettudományi Kutatóközpont. The sequence listing filed with the application follows.

SEQUENCE LISTING (12 sequences)

SEQ ID NO: 1 - protein, 10 aa, Homo sapiens
KAPIISGVTK

SEQ ID NO: 2 - protein, 15 aa, Homo sapiens
EMPSEEGYQDYEPEA

SEQ ID NO: 3 - protein, 131 aa, Homo sapiens
ASPELSALEEAFRRFAVHGDARATGREMHGKNWSKLCKDCQVIDGRNVTVTDVDIVFSKIKGKSCRTITFEQFQEALEELAKKRFKDKSSEEAVREVHRLIEGKAPIISGVTKAISSPTVSRLTDTTKFTG

SEQ ID NO: 4 - protein, 20 aa, Homo sapiens
DNEAYEMPSEEGYQDYEPEA

SEQ ID NO: 5 - protein, 45 aa, Homo sapiens
KKDHMGKGEEGASQEGILEDMPVDPDNEAYEMPSEEGYQDYEPEA

SEQ ID NO: 6 - protein, 219 aa, Homo sapiens
MADKAKPAKAANRTPPKSPGDPSKDRAAKRLSLESEGAGEGAAASPELSALEEAFRRFAVHGDARATGREMHGKNWSKLCKDCQVIDGRNVTVTDVDIVFSKIKGKSCRTITFEQFQEALEELAKKRFKDKSSEEAVREVHRLIEGKAPIISGVTKAISSPTVSRLTDTTKFTGSHKERFDPSGKGKGKAGRVDLVDESGYVSGYKHAGTYDQKVQGGK

SEQ ID NO: 7 - protein, 140 aa, Homo sapiens
MDVFMKGLSKAKEGVVAAAEKTKQGVAEAAGRTKEGVLYVGSKTKEGVVHGVTTVAEKTKEQVTNVGEAVVTGVTAVAQKTVEGAGSIAAATGFGKKDHMGKGEEGASQEGILEDMPVDPDNEAYEMPSEEGYQDYEPEA

SEQ ID NO: 8 - protein, 4 aa, Homo sapiens
AVHG

SEQ ID NO: 9 - protein, 5 aa, Homo sapiens
SGVTK

SEQ ID NO: 10 - protein, 10 aa, Homo sapiens
RLIEGKAPII

SEQ ID NO: 11 - DNA, 37 bp, synthetic construct
  source 1..37: mol_type = other DNA
gaaggagatatacatatggatgtattcatgaaaggac

SEQ ID NO: 12 - DNA, 71 bp, synthetic construct
  source 1..71: mol_type = other DNA
atatctcgagggcttcaggttccgtagtcttgatacccttcctcatcaggcatttcataagcctcattgtc